European Patent Specification EP 4 409 297 B1, published January 29, 2025. Title: Novel method for determining a concentration of N-terminal pro-hormone BNP (NT-proBNP) in a sample. Applicant: GENTIAN AS. The sequence listing filed with the application follows.

SEQUENCE LISTING (13 sequences)

SEQ ID NO: 1 - protein, 76 aa, Homo sapiens
HPLGSPGSASDLETSGLQEQRNHLQGKLSELQVEQTSLEPLQESPRPTGVWKSREVATEGIRGHRKMVLYTLRAPR

SEQ ID NO: 2 - protein, 26 aa, Homo sapiens
SASDLETSGLQEQRNHLQGKLSELQV

SEQ ID NO: 3 - protein, 14 aa, Homo sapiens
IRGHRKMVLYTLRA

SEQ ID NO: 4 - protein, 5 aa, synthetic construct
SASDL

SEQ ID NO: 5 - protein, 14 aa, synthetic construct
DLETSGLQEQRNHL

SEQ ID NO: 6 - protein, 7 aa, synthetic construct
NHLQGKL

SEQ ID NO: 7 - protein, 8 aa, synthetic construct
SASDLETS

SEQ ID NO: 8 - protein, 6 aa, synthetic construct
ETSGLQ

SEQ ID NO: 9 - protein, 7 aa, synthetic construct
GKLSELQ

SEQ ID NO: 10 - protein, 6 aa, synthetic construct
GLQEQR

SEQ ID NO: 11 - protein, 6 aa, synthetic construct
NHLQGK

SEQ ID NO: 12 - protein, 8 aa, synthetic construct
EVATEGIR

SEQ ID NO: 13 - protein, 7 aa, synthetic construct
MVLYTLR